European Patent Application EP 4 155 400 A1, published March 29, 2023. Title: UDP-GLYCOSYLTRANSFERASES. Applicant: DSM IP Assets B.V. Application EP. The sequence listing filed with the application follows.

SEQUENCE LISTING (34 sequences)

SEQ ID NO: 1 - DNA, 1383 bp, Stevia rebaudiana
  source 1..1383: mol_type = genomic DNA
atggccgagcagcagaagatcaagaagtctccccacgttctgctcatccccttccctctgcagggccacatcaaccccttcatccagttcggcaagcgactcatctccaagggtgtcaagaccactctggtcaccaccatccacaccctcaactccactctcaaccactccaacaccaccaccacctccatcgagatccaggccatctccgacggctgtgacgagggtggtttcatgtctgctggtgagtcttacctcgagactttcaagcaggtcggttccaagtctctggctgacctcatcaagaagctccagtccgagggtaccaccattgacgccatcatctacgactccatgaccgagtgggttctcgatgtcgccatcgagtttggtattgacggtggctccttcttcacccaggcctgtgtcgtcaactctctctactaccacgtccacaagggtctgatctctctgcccctcggcgagactgtctccgtccccggtttccccgttctgcagcgatgggagactcctctcattctccagaaccacgagcagatccagtccccctggtcccagatgctcttcggccagttcgccaacattgaccaggcccgatgggttttcaccaactccttctacaagctcgaggaagaggtcattgagtggacccgaaagatctggaacctcaaggtcattggccccaccctcccctccatgtacctcgacaagcgactcgatgacgacaaggacaacggtttcaacctctacaaggccaaccaccacgagtgcatgaactggctcgacgacaagcccaaggagtccgttgtctacgttgcctttggctctctggtcaagcacggccccgagcaggttgaggagatcacccgagctctgattgactccgatgtcaacttcctgtgggtcatcaagcacaaggaagagggtaagctccccgagaacctgtccgaggtcatcaagaccggcaagggcctcattgttgcctggtgcaagcagctcgacgttctcgcccacgagtccgtcggctgctttgtcacccactgcggtttcaactccaccctcgaggctatctctctcggtgtccccgttgttgccatgccccagttctccgaccagaccaccaacgccaagctcctcgatgagattctcggtgtcggtgtccgagtcaaggctgacgagaacggtattgtccgacgaggtaacctggcttcttgtatcaagatgatcatggaggaagagcgaggtgtcatcatccgaaagaacgccgtcaagtggaaggatctggccaaggttgctgtccacgagggtggctcttccgacaacgacattgtcgagtttgtctccgagctcatcaaggcctaa

SEQ ID NO: 2 - protein, 460 aa, Stevia rebaudiana
  SOURCE 1..460
MAEQQKIKKSPHVLLIPFPLQGHINPFIQFGKRLISKGVKTTLVTTIHTLNSTLNHSNTTTTSIEIQAISDGCDEGGFMSAGESYLETFKQVGSKSLADLIKKLQSEGTTIDAIIYDSMTEWVLDVAIEFGIDGGSFFTQACVVNSLYYHVHKGLISLPLGETVSVPGFPVLQRWETPLILQNHEQIQSPWSQMLFGQFANIDQARWVFTNSFYKLEEEVIEWTRKIWNLKVIGPTLPSMYLDKRLDDDKDNGFNLYKANHHECMNWLDDKPKESVVYVAFGSLVKHGPEQVEEITRALIDSDVNFLWVIKHKEEGKLPENLSEVIKTGKGLIVAWCKQLDVLAHESVGCFVTHCGFNSTLEAISLGVPVVAMPQFSDQTTNAKLLDEILGVGVRVKADENGIVRRGNLASCIKMIMEEERGVIIRKNAVKWKDLAKVAVHEGGSSDNDIVEFVSELIKA

SEQ ID NO: 3 - DNA, 1383 bp, synthetic construct
  source 1..1383: mol_type = other DNA
  misc_feature 1..1383: note = UDP-glycosyltransferase variant encoding sequence
atggccgagcagcagaagatcaagaagtctccccacgttctgctcatccccttccctctgcagggccacatcaaccccttcatccagttcggcaagcgactcgtctccaagggtgtcaagaccactctggtcaccaccatccacaccctcaactccactctcaaccactccaacaccaccaccacctccatcgagatccaggccatctccgacggctgtgacgagggtggtttcatgtctgctggtgagtcttacctcgagactttcaagcaggtcggttccaagtctctggctgacctcatcaagaagctccagtccgagggtaccaccattgacgccatcatctacgactccatgaccgagtgggttctcgatgtcgccatcgagtttggtattgacggtggctccttcttcacccaggcctgtgtcgtcaactctctctactaccacgtccacaagggtctgatctctctgcccctcggcgagactgtctccgtccccggtttccccgttctgcagcgatgggagactcctctcattctccagaaccacgagcagatccagtccccctggtcccagatgctcttcggccagttcgccaacattgaccaggcccgatgggttttcaccaactccttctacaagctcgaggaagaggtcattgagtggacccgaaagatctggaacctcaaggtcattggccccaccctcccctccatgtacctcgacaagcgactcgatgacgacaaggacaacggtttcaacctctacaaggccaaccaccacgagtgcatgaactggctcgacgacaagcccaaggagtccgttgtctacgttgcctttggctctctggtcaagcacggccccgagcaggttgaggagatcacccgagctctgattgactccgatgtcaacttcctgtgggtcatcaagcacaaggaagagggtaagctccccgagaacctgtccgaggtcatcaagaccggcaagggcctcattgttgcctggtgcaagcagctcgacgttctcgcccacgagtccgtcggctgctttgtcacccactgcggtttcaactccaccctcgaggctatctctctcggtgtccccgttgttgccatgccccagttctccgaccagaccaccaacgccaagctcctcgatgagattctcggtgtcggtgtccgagtcaaggctgacgagaacggtattgtccgacgaggtaacctggcttcttgtatcaagatgatcatggaggaagagcgaggtgtcatcatccgaaagaacgccgtcaagtggaaggatctggccaaggttgctgtccacgagggtggctcttccgacaacgacattgtcgagtttgtctccgagctcatcaaggcctaa

SEQ ID NO: 4 - protein, 460 aa, synthetic construct
  SOURCE 1..460
  VARIANT 1..460: NOTE = UDP-glycosyltransferase variant
MAEQQKIKKSPHVLLIPFPLQGHINPFIQFGKRLVSKGVKTTLVTTIHTLNSTLNHSNTTTTSIEIQAISDGCDEGGFMSAGESYLETFKQVGSKSLADLIKKLQSEGTTIDAIIYDSMTEWVLDVAIEFGIDGGSFFTQACVVNSLYYHVHKGLISLPLGETVSVPGFPVLQRWETPLILQNHEQIQSPWSQMLFGQFANIDQARWVFTNSFYKLEEEVIEWTRKIWNLKVIGPTLPSMYLDKRLDDDKDNGFNLYKANHHECMNWLDDKPKESVVYVAFGSLVKHGPEQVEEITRALIDSDVNFLWVIKHKEEGKLPENLSEVIKTGKGLIVAWCKQLDVLAHESVGCFVTHCGFNSTLEAISLGVPVVAMPQFSDQTTNAKLLDEILGVGVRVKADENGIVRRGNLASCIKMIMEEERGVIIRKNAVKWKDLAKVAVHEGGSSDNDIVEFVSELIKA

SEQ ID NO: 5 - DNA, 1383 bp, synthetic construct
  source 1..1383: mol_type = other DNA
  misc_feature 1..1383: note = UDP-glycosyltransferase variant encoding sequence
atggccgagcagcagaagatcaagaagtctccccacgttctgctcatccccttccctctgcagggccacatcaaccccttcatccagttcggcaagcgactcatctccaagggtgtcaagaccactctggtcaccaccatccacaccctcaactccactctcaaccactccaacaccaccaccacctccatcgagatccaggccatctccgacggctgtgacgagggtggtttcatgtctgctggtgagtcttacctcgagactttcaagcaggtcggttccaagtctctggctgacctcatcaagaagctccagtccgagggtaccaccattgacgccatcatctacgactccatgaccgagtgggttctcgatgtcgccatcgagtttggtattgacggtggctccttcttcacccaggcctgtgtcgtcaactctctctactaccacgtccacaagggtctgatctctctgcccctcggcgagactgtctccgtccccggtttccccgttctgcagcgatgggagactcctctcattctccagaaccacgagcagatccaggccccctggtcccagatgctcttcggccagttcgccaacattgaccaggcccgatgggttttcaccaactccttctacaagctcgaggaagaggtcattgagtggacccgaaagatctggaacctcaaggtcattggccccaccctcccctccatgtacctcgacaagcgactcgatgacgacaaggacaacggtttcaacctctacaaggccaaccaccacgagtgcatgaactggctcgacgacaagcccaaggagtccgttgtctacgttgcctttggctctctggtcaagcacggccccgagcaggttgaggagatcacccgagctctgattgactccgatgtcaacttcctgtgggtcatcaagcacaaggaagagggtaagctccccgagaacctgtccgaggtcatcaagaccggcaagggcctcattgttgcctggtgcaagcagctcgacgttctcgcccacgagtccgtcggctgctttgtcacccactgcggtttcaactccaccctcgaggctatctctctcggtgtccccgttgttgccatgccccagttctccgaccagaccaccaacgccaagctcctcgatgagattctcggtgtcggtgtccgagtcaaggctgacgagaacggtattgtccgacgaggtaacctggcttcttgtatcaagatgatcatggaggaagagcgaggtgtcatcatccgaaagaacgccgtcaagtggaaggatctggccaaggttgctgtccacgagggtggctcttccgacaacgacattgtcgagtttgtctccgagctcatcaaggcctaa

SEQ ID NO: 6 - protein, 460 aa, synthetic construct
  SOURCE 1..460
  VARIANT 1..460: NOTE = UDP-glycosyltransferase variant
MAEQQKIKKSPHVLLIPFPLQGHINPFIQFGKRLISKGVKTTLVTTIHTLNSTLNHSNTTTTSIEIQAISDGCDEGGFMSAGESYLETFKQVGSKSLADLIKKLQSEGTTIDAIIYDSMTEWVLDVAIEFGIDGGSFFTQACVVNSLYYHVHKGLISLPLGETVSVPGFPVLQRWETPLILQNHEQIQAPWSQMLFGQFANIDQARWVFTNSFYKLEEEVIEWTRKIWNLKVIGPTLPSMYLDKRLDDDKDNGFNLYKANHHECMNWLDDKPKESVVYVAFGSLVKHGPEQVEEITRALIDSDVNFLWVIKHKEEGKLPENLSEVIKTGKGLIVAWCKQLDVLAHESVGCFVTHCGFNSTLEAISLGVPVVAMPQFSDQTTNAKLLDEILGVGVRVKADENGIVRRGNLASCIKMIMEEERGVIIRKNAVKWKDLAKVAVHEGGSSDNDIVEFVSELIKA

SEQ ID NO: 7 - DNA, 1383 bp, synthetic construct
  source 1..1383: mol_type = other DNA
  misc_feature 1..1383: note = UDP-glycosyltransferase variant encoding sequence
atggccgagcagcagaagatcaagaagtctccccacgttctgctcatccccttccctctgcagggccacatcaaccccttcatccagttcggcaagcgactcatctccaagggtgtcaagaccactctggtcaccaccatccacaccctcaactccactctcaaccactccaacaccaccaccacctccatcgagatccaggccatctccgacggctgtgacgagggtggtttcatgtctgctggtgagtcttacctcgagactttcaagcaggtcggttccaagtctctggctgacctcatcaagaagctccagtccgagggtaccaccattgacgccatcatctacgactccatgaccgagtgggttctcgatgtcgccatcgagtttggtattgacggtggctccttcttcacccaggcctgtgtcgtcaactctctctactaccacgtccacaagggtctgatctctctgcccctcggcgagactgtctccgtccccggtttccccgttctgcagcgatgggagactcctctcattctccagaaccacgagcagatccagtccccctggtcccagatgctcttcggccagttcgccaacattgaccaggcccgatgggttttcaccaactccttctacaagctcgaggaagaggtcattgagtggacccgaaagatctggaacctcaaggtcattggccccaccctcccctccatgtacctcgacaagcgactcgatgacgacaaggacaacggtttcaacctctacaaggccaaccaccacgagtgcatgaactggctcgacgacaagcccaaggagtccgttgtctacgttaactttggctctctggtcaagcacggccccgagcaggttgaggagatcacccgagctctgattgactccgatgtcaacttcctgtgggtcatcaagcacaaggaagagggtaagctccccgagaacctgtccgaggtcatcaagaccggcaagggcctcattgttgcctggtgcaagcagctcgacgttctcgcccacgagtccgtcggctgctttgtcacccactgcggtttcaactccaccctcgaggctatctctctcggtgtccccgttgttgccatgccccagttctccgaccagaccaccaacgccaagctcctcgatgagattctcggtgtcggtgtccgagtcaaggctgacgagaacggtattgtccgacgaggtaacctggcttcttgtatcaagatgatcatggaggaagagcgaggtgtcatcatccgaaagaacgccgtcaagtggaaggatctggccaaggttgctgtccacgagggtggctcttccgacaacgacattgtcgagtttgtctccgagctcatcaaggcctaa

SEQ ID NO: 8 - protein, 460 aa, synthetic construct
  SOURCE 1..460
  VARIANT 1..460: NOTE = UDP-glycosyltransferase variant
MAEQQKIKKSPHVLLIPFPLQGHINPFIQFGKRLISKGVKTTLVTTIHTLNSTLNHSNTTTTSIEIQAISDGCDEGGFMSAGESYLETFKQVGSKSLADLIKKLQSEGTTIDAIIYDSMTEWVLDVAIEFGIDGGSFFTQACVVNSLYYHVHKGLISLPLGETVSVPGFPVLQRWETPLILQNHEQIQSPWSQMLFGQFANIDQARWVFTNSFYKLEEEVIEWTRKIWNLKVIGPTLPSMYLDKRLDDDKDNGFNLYKANHHECMNWLDDKPKESVVYVNFGSLVKHGPEQVEEITRALIDSDVNFLWVIKHKEEGKLPENLSEVIKTGKGLIVAWCKQLDVLAHESVGCFVTHCGFNSTLEAISLGVPVVAMPQFSDQTTNAKLLDEILGVGVRVKADENGIVRRGNLASCIKMIMEEERGVIIRKNAVKWKDLAKVAVHEGGSSDNDIVEFVSELIKA

SEQ ID NO: 9 - DNA, 1383 bp, synthetic construct
  source 1..1383: mol_type = other DNA
  misc_feature 1..1383: note = UDP-glycosyltransferase variant encoding sequence
atggccgagcagcagaagatcaagaagtctccccacgttctgctcatccccttccctctgcagggccacatcaaccccttcatccagttcggcaagcgactcatctccaagggtgtcaagaccactctggtcaccaccatccacaccctcaactccactctcaaccactccaacaccaccaccacctccatcgagatccaggccatctccgacggctgtgacgagggtggtttcatgtctgctggtgagtcttacctcgagactttcaagcaggtcggttccaagtctctggctgacctcatcaagaagctccagtccgagggtaccaccattgacgccatcatctacgactccatgaccgagtgggttctcgatgtcgccatcgagtttggtattgacggtggctccttcttcacccaggcctgtgtcgtcaactctctctactaccacgtccacaagggtctgatctctctgcccctcggcgagactgtctccgtccccggtttccccgttctgcagcgatgggagactcctctcattctccagaaccacgagcagatccagtccccctggtcccagatgctcttcggccagttcgccaacattgaccaggcccgatgggttttcaccaactccttctacaagctcgaggaagaggtcattgagtggacccgaaagatctggaacctcaaggtcattggccccaccctcccctccatgtacctcgacaagcgactcgatgacgacaaggacaacggtttcaacctctacaaggccaaccaccacgagtgcatgaactggctcgacgacaagcccaaggagtccgttgtctacgttgcctttggctctaacgtcaagcacggccccgagcaggttgaggagatcacccgagctctgattgactccgatgtcaacttcctgtgggtcatcaagcacaaggaagagggtaagctccccgagaacctgtccgaggtcatcaagaccggcaagggcctcattgttgcctggtgcaagcagctcgacgttctcgcccacgagtccgtcggctgctttgtcacccactgcggtttcaactccaccctcgaggctatctctctcggtgtccccgttgttgccatgccccagttctccgaccagaccaccaacgccaagctcctcgatgagattctcggtgtcggtgtccgagtcaaggctgacgagaacggtattgtccgacgaggtaacctggcttcttgtatcaagatgatcatggaggaagagcgaggtgtcatcatccgaaagaacgccgtcaagtggaaggatctggccaaggttgctgtccacgagggtggctcttccgacaacgacattgtcgagtttgtctccgagctcatcaaggcctaa

SEQ ID NO: 10 - protein, 460 aa, synthetic construct
  SOURCE 1..460
  VARIANT 1..460: NOTE = UDP-glycosyltransferase variant
MAEQQKIKKSPHVLLIPFPLQGHINPFIQFGKRLISKGVKTTLVTTIHTLNSTLNHSNTTTTSIEIQAISDGCDEGGFMSAGESYLETFKQVGSKSLADLIKKLQSEGTTIDAIIYDSMTEWVLDVAIEFGIDGGSFFTQACVVNSLYYHVHKGLISLPLGETVSVPGFPVLQRWETPLILQNHEQIQSPWSQMLFGQFANIDQARWVFTNSFYKLEEEVIEWTRKIWNLKVIGPTLPSMYLDKRLDDDKDNGFNLYKANHHECMNWLDDKPKESVVYVAFGSNVKHGPEQVEEITRALIDSDVNFLWVIKHKEEGKLPENLSEVIKTGKGLIVAWCKQLDVLAHESVGCFVTHCGFNSTLEAISLGVPVVAMPQFSDQTTNAKLLDEILGVGVRVKADENGIVRRGNLASCIKMIMEEERGVIIRKNAVKWKDLAKVAVHEGGSSDNDIVEFVSELIKA

SEQ ID NO: 11 - DNA, 1383 bp, synthetic construct
  source 1..1383: mol_type = other DNA
  misc_feature 1..1383: note = UDP-glycosyltransferase variant encoding sequence
atggccgagcagcagaagatcaagaagtctccccacgttctgctcatccccttccctctgcagggccacatcaaccccttcatccagttcggcaagcgactcatctccaagggtgtcaagaccactctggtcaccaccatccacaccctcaactccactctcaaccactccaacaccaccaccacctccatcgagatccaggccatctccgacggctgtgacgagggtggtttcatgtctgctggtgagtcttacctcgagactttcaagcaggtcggttccaagtctctggctgacctcatcaagaagctccagtccgagggtaccaccattgacgccatcatctacgactccatgaccgagtgggttctcgatgtcgccatcgagtttggtattgacggtggctccttcttcacccaggcctgtgtcgtcaactctctctactaccacgtccacaagggtctgatctctctgcccctcggcgagactgtctccgtccccggtttccccgttctgcagcgatgggagactcctctcattctccagaaccacgagcagatccagtccccctggtcccagatgctcttcggccagttcgccaacattgaccaggcccgatgggttttcaccaactccttctacaagctcgaggaagaggtcattgagtggacccgaaagatctggaacctcaaggtcattggccccaccctcccctccatgtacctcgacaagcgactcgatgacgacaaggacaacggtttcaacctctacaaggccaaccaccacgagtgcatgaactggctcgacgacaagcccaaggagtccgttgtctacgttgcctttggctctctgggcaagcacggccccgagcaggttgaggagatcacccgagctctgattgactccgatgtcaacttcctgtgggtcatcaagcacaaggaagagggtaagctccccgagaacctgtccgaggtcatcaagaccggcaagggcctcattgttgcctggtgcaagcagctcgacgttctcgcccacgagtccgtcggctgctttgtcacccactgcggtttcaactccaccctcgaggctatctctctcggtgtccccgttgttgccatgccccagttctccgaccagaccaccaacgccaagctcctcgatgagattctcggtgtcggtgtccgagtcaaggctgacgagaacggtattgtccgacgaggtaacctggcttcttgtatcaagatgatcatggaggaagagcgaggtgtcatcatccgaaagaacgccgtcaagtggaaggatctggccaaggttgctgtccacgagggtggctcttccgacaacgacattgtcgagtttgtctccgagctcatcaaggcctaa

SEQ ID NO: 12 - protein, 460 aa, synthetic construct
  SOURCE 1..460
  VARIANT 1..460: NOTE = UDP-glycosyltransferase variant
MAEQQKIKKSPHVLLIPFPLQGHINPFIQFGKRLISKGVKTTLVTTIHTLNSTLNHSNTTTTSIEIQAISDGCDEGGFMSAGESYLETFKQVGSKSLADLIKKLQSEGTTIDAIIYDSMTEWVLDVAIEFGIDGGSFFTQACVVNSLYYHVHKGLISLPLGETVSVPGFPVLQRWETPLILQNHEQIQSPWSQMLFGQFANIDQARWVFTNSFYKLEEEVIEWTRKIWNLKVIGPTLPSMYLDKRLDDDKDNGFNLYKANHHECMNWLDDKPKESVVYVAFGSLGKHGPEQVEEITRALIDSDVNFLWVIKHKEEGKLPENLSEVIKTGKGLIVAWCKQLDVLAHESVGCFVTHCGFNSTLEAISLGVPVVAMPQFSDQTTNAKLLDEILGVGVRVKADENGIVRRGNLASCIKMIMEEERGVIIRKNAVKWKDLAKVAVHEGGSSDNDIVEFVSELIKA

SEQ ID NO: 13 - DNA, 1383 bp, synthetic construct
  source 1..1383: mol_type = other DNA
  misc_feature 1..1383: note = UDP-glycosyltransferase variant encoding sequence
atggccgagcagcagaagatcaagaagtctccccacgttctgctcatccccttccctctgcagggccacatcaaccccttcatccagttcggcaagcgactcatctccaagggtgtcaagaccactctggtcaccaccatccacaccctcaactccactctcaaccactccaacaccaccaccacctccatcgagatccaggccatctccgacggctgtgacgagggtggtttcatgtctgctggtgagtcttacctcgagactttcaagcaggtcggttccaagtctctggctgacctcatcaagaagctccagtccgagggtaccaccattgacgccatcatctacgactccatgaccgagtgggttctcgatgtcgccatcgagtttggtattgacggtggctccttcttcacccaggcctgtgtcgtcaactctctctactaccacgtccacaagggtctgatctctctgcccctcggcgagactgtctccgtccccggtttccccgttctgcagcgatgggagactcctctcattctccagaaccacgagcagatccagtccccctggtcccagatgctcttcggccagttcgccaacattgaccaggcccgatgggttttcaccaactccttctacaagctcgaggaagaggtcattgagtggacccgaaagatctggaacctcaaggtcattggccccaccctcccctccatgtacctcgacaagcgactcgatgacgacaaggacaacggtttcaacctctacaaggccaaccaccacgagtgcatgaactggctcgacgacaagcccaaggagtccgttgtctacgttgcctttggctctctgaacaagcacggccccgagcaggttgaggagatcacccgagctctgattgactccgatgtcaacttcctgtgggtcatcaagcacaaggaagagggtaagctccccgagaacctgtccgaggtcatcaagaccggcaagggcctcattgttgcctggtgcaagcagctcgacgttctcgcccacgagtccgtcggctgctttgtcacccactgcggtttcaactccaccctcgaggctatctctctcggtgtccccgttgttgccatgccccagttctccgaccagaccaccaacgccaagctcctcgatgagattctcggtgtcggtgtccgagtcaaggctgacgagaacggtattgtccgacgaggtaacctggcttcttgtatcaagatgatcatggaggaagagcgaggtgtcatcatccgaaagaacgccgtcaagtggaaggatctggccaaggttgctgtccacgagggtggctcttccgacaacgacattgtcgagtttgtctccgagctcatcaaggcctaa

SEQ ID NO: 14 - protein, 460 aa, synthetic construct
  SOURCE 1..460
  VARIANT 1..460: NOTE = UDP-glycosyltransferase variant
MAEQQKIKKSPHVLLIPFPLQGHINPFIQFGKRLISKGVKTTLVTTIHTLNSTLNHSNTTTTSIEIQAISDGCDEGGFMSAGESYLETFKQVGSKSLADLIKKLQSEGTTIDAIIYDSMTEWVLDVAIEFGIDGGSFFTQACVVNSLYYHVHKGLISLPLGETVSVPGFPVLQRWETPLILQNHEQIQSPWSQMLFGQFANIDQARWVFTNSFYKLEEEVIEWTRKIWNLKVIGPTLPSMYLDKRLDDDKDNGFNLYKANHHECMNWLDDKPKESVVYVAFGSLNKHGPEQVEEITRALIDSDVNFLWVIKHKEEGKLPENLSEVIKTGKGLIVAWCKQLDVLAHESVGCFVTHCGFNSTLEAISLGVPVVAMPQFSDQTTNAKLLDEILGVGVRVKADENGIVRRGNLASCIKMIMEEERGVIIRKNAVKWKDLAKVAVHEGGSSDNDIVEFVSELIKA

SEQ ID NO: 15 - DNA, 1383 bp, synthetic construct
  source 1..1383: mol_type = other DNA
  misc_feature 1..1383: note = UDP-glycosyltransferase variant encoding sequence
atggccgagcagcagaagatcaagaagtctccccacgttctgctcatccccttccctctgcagggccacatcaaccccttcatccagttcggcaagcgactcatctccaagggtgtcaagaccactctggtcaccaccatccacaccctcaactccactctcaaccactccaacaccaccaccacctccatcgagatccaggccatctccgacggctgtgacgagggtggtttcatgtctgctggtgagtcttacctcgagactttcaagcaggtcggttccaagtctctggctgacctcatcaagaagctccagtccgagggtaccaccattgacgccatcatctacgactccatgaccgagtgggttctcgatgtcgccatcgagtttggtattgacggtggctccttcttcacccaggcctgtgtcgtcaactctctctactaccacgtccacaagggtctgatctctctgcccctcggcgagactgtctccgtccccggtttccccgttctgcagcgatgggagactcctctcattctccagaaccacgagcagatccagtccccctggtcccagatgctcttcggccagttcgccaacattgaccaggcccgatgggttttcaccaactccttctacaagctcgaggaagaggtcattgagtggacccgaaagatctggaacctcaaggtcattggccccaccctcccctccatgtacctcgacaagcgactcgatgacgacaaggacaacggtttcaacctctacaaggccaaccaccacgagtgcatgaactggctcgacgacaagcccaaggagtccgttgtctacgttgcctttggctctctgtccaagcacggccccgagcaggttgaggagatcacccgagctctgattgactccgatgtcaacttcctgtgggtcatcaagcacaaggaagagggtaagctccccgagaacctgtccgaggtcatcaagaccggcaagggcctcattgttgcctggtgcaagcagctcgacgttctcgcccacgagtccgtcggctgctttgtcacccactgcggtttcaactccaccctcgaggctatctctctcggtgtccccgttgttgccatgccccagttctccgaccagaccaccaacgccaagctcctcgatgagattctcggtgtcggtgtccgagtcaaggctgacgagaacggtattgtccgacgaggtaacctggcttcttgtatcaagatgatcatggaggaagagcgaggtgtcatcatccgaaagaacgccgtcaagtggaaggatctggccaaggttgctgtccacgagggtggctcttccgacaacgacattgtcgagtttgtctccgagctcatcaaggcctaa

SEQ ID NO: 16 - protein, 460 aa, synthetic construct
  SOURCE 1..460
  VARIANT 1..460: NOTE = UDP-glycosyltransferase variant
MAEQQKIKKSPHVLLIPFPLQGHINPFIQFGKRLISKGVKTTLVTTIHTLNSTLNHSNTTTTSIEIQAISDGCDEGGFMSAGESYLETFKQVGSKSLADLIKKLQSEGTTIDAIIYDSMTEWVLDVAIEFGIDGGSFFTQACVVNSLYYHVHKGLISLPLGETVSVPGFPVLQRWETPLILQNHEQIQSPWSQMLFGQFANIDQARWVFTNSFYKLEEEVIEWTRKIWNLKVIGPTLPSMYLDKRLDDDKDNGFNLYKANHHECMNWLDDKPKESVVYVAFGSLSKHGPEQVEEITRALIDSDVNFLWVIKHKEEGKLPENLSEVIKTGKGLIVAWCKQLDVLAHESVGCFVTHCGFNSTLEAISLGVPVVAMPQFSDQTTNAKLLDEILGVGVRVKADENGIVRRGNLASCIKMIMEEERGVIIRKNAVKWKDLAKVAVHEGGSSDNDIVEFVSELIKA

SEQ ID NO: 17 - DNA, 1383 bp, synthetic construct
  source 1..1383: mol_type = other DNA
  misc_feature 1..1383: note = UDP-glycosyltransferase variant encoding sequence
atggccgagcagcagaagatcaagaagtctccccacgttctgctcatccccttccctctgcagggccacatcaaccccttcatccagttcggcaagcgactcatctccaagggtgtcaagaccactctggtcaccaccatccacaccctcaactccactctcaaccactccaacaccaccaccacctccatcgagatccaggccatctccgacggctgtgacgagggtggtttcatgtctgctggtgagtcttacctcgagactttcaagcaggtcggttccaagtctctggctgacctcatcaagaagctccagtccgagggtaccaccattgacgccatcatctacgactccatgaccgagtgggttctcgatgtcgccatcgagtttggtattgacggtggctccttcttcacccaggcctgtgtcgtcaactctctctactaccacgtccacaagggtctgatctctctgcccctcggcgagactgtctccgtccccggtttccccgttctgcagcgatgggagactcctctcattctccagaaccacgagcagatccagtccccctggtcccagatgctcttcggccagttcgccaacattgaccaggcccgatgggttttcaccaactccttctacaagctcgaggaagaggtcattgagtggacccgaaagatctggaacctcaaggtcattggccccaccctcccctccatgtacctcgacaagcgactcgatgacgacaaggacaacggtttcaacctctacaaggccaaccaccacgagtgcatgaactggctcgacgacaagcccaaggagtccgttgtctacgttgcctttggctctctggtcaagcacggccccgagcaggttgaggagatcacccgagctctgattgactccgatgtcaacttcctgtgggtcatcaagcacaaggaagagggtaagctccccgagaacctgtccgaggtcatcaagaccggcaagggcctcattgctgcctggtgcaagcagctcgacgttctcgcccacgagtccgtcggctgctttgtcacccactgcggtttcaactccaccctcgaggctatctctctcggtgtccccgttgttgccatgccccagttctccgaccagaccaccaacgccaagctcctcgatgagattctcggtgtcggtgtccgagtcaaggctgacgagaacggtattgtccgacgaggtaacctggcttcttgtatcaagatgatcatggaggaagagcgaggtgtcatcatccgaaagaacgccgtcaagtggaaggatctggccaaggttgctgtccacgagggtggctcttccgacaacgacattgtcgagtttgtctccgagctcatcaaggcctaa

SEQ ID NO: 18 - protein, 460 aa, synthetic construct
  SOURCE 1..460
  VARIANT 1..460: NOTE = UDP-glycosyltransferase variant
MAEQQKIKKSPHVLLIPFPLQGHINPFIQFGKRLISKGVKTTLVTTIHTLNSTLNHSNTTTTSIEIQAISDGCDEGGFMSAGESYLETFKQVGSKSLADLIKKLQSEGTTIDAIIYDSMTEWVLDVAIEFGIDGGSFFTQACVVNSLYYHVHKGLISLPLGETVSVPGFPVLQRWETPLILQNHEQIQSPWSQMLFGQFANIDQARWVFTNSFYKLEEEVIEWTRKIWNLKVIGPTLPSMYLDKRLDDDKDNGFNLYKANHHECMNWLDDKPKESVVYVAFGSLVKHGPEQVEEITRALIDSDVNFLWVIKHKEEGKLPENLSEVIKTGKGLIAAWCKQLDVLAHESVGCFVTHCGFNSTLEAISLGVPVVAMPQFSDQTTNAKLLDEILGVGVRVKADENGIVRRGNLASCIKMIMEEERGVIIRKNAVKWKDLAKVAVHEGGSSDNDIVEFVSELIKA

SEQ ID NO: 19 - DNA, 1383 bp, synthetic construct
  source 1..1383: mol_type = other DNA
  misc_feature 1..1383: note = UDP-glycosyltransferase variant encoding sequence
atggccgagcagcagaagatcaagaagtctccccacgttctgctcatccccttccctctgcagggccacatcaaccccttcatccagttcggcaagcgactcatctccaagggtgtcaagaccactctggtcaccaccatccacaccctcaactccactctcaaccactccaacaccaccaccacctccatcgagatccaggccatctccgacggctgtgacgagggtggtttcatgtctgctggtgagtcttacctcgagactttcaagcaggtcggttccaagtctctggctgacctcatcaagaagctccagtccgagggtaccaccattgacgccatcatctacgactccatgaccgagtgggttctcgatgtcgccatcgagtttggtattgacggtggctccttcttcacccaggcctgtgtcgtcaactctctctactaccacgtccacaagggtctgatctctctgcccctcggcgagactgtctccgtccccggtttccccgttctgcagcgatgggagactcctctcattctccagaaccacgagcagatccagtccccctggtcccagatgctcttcggccagttcgccaacattgaccaggcccgatgggttttcaccaactccttctacaagctcgaggaagaggtcattgagtggacccgaaagatctggaacctcaaggtcattggccccaccctcccctccatgtacctcgacaagcgactcgatgacgacaaggacaacggtttcaacctctacaaggccaaccaccacgagtgcatgaactggctcgacgacaagcccaaggagtccgttgtctacgttgcctttggctctctggtcaagcacggccccgagcaggttgaggagatcacccgagctctgattgactccgatgtcaacttcctgtgggtcatcaagcacaaggaagagggtaagctccccgagaacctgtccgaggtcatcaagaccggcaagggcctcattgttgcctggtgcaagcagctcgacgttctcgcccacgagtccgtcggctgctttgtcacccactgcggtttcaactccaccctcgaggctatctctctcggtgtccccgttgttgccgccccccagttctccgaccagaccaccaacgccaagctcctcgatgagattctcggtgtcggtgtccgagtcaaggctgacgagaacggtattgtccgacgaggtaacctggcttcttgtatcaagatgatcatggaggaagagcgaggtgtcatcatccgaaagaacgccgtcaagtggaaggatctggccaaggttgctgtccacgagggtggctcttccgacaacgacattgtcgagtttgtctccgagctcatcaaggcctaa

SEQ ID NO: 20 - protein, 460 aa, synthetic construct
  SOURCE 1..460
  VARIANT 1..460: NOTE = UDP-glycosyltransferase variant
MAEQQKIKKSPHVLLIPFPLQGHINPFIQFGKRLISKGVKTTLVTTIHTLNSTLNHSNTTTTSIEIQAISDGCDEGGFMSAGESYLETFKQVGSKSLADLIKKLQSEGTTIDAIIYDSMTEWVLDVAIEFGIDGGSFFTQACVVNSLYYHVHKGLISLPLGETVSVPGFPVLQRWETPLILQNHEQIQSPWSQMLFGQFANIDQARWVFTNSFYKLEEEVIEWTRKIWNLKVIGPTLPSMYLDKRLDDDKDNGFNLYKANHHECMNWLDDKPKESVVYVAFGSLVKHGPEQVEEITRALIDSDVNFLWVIKHKEEGKLPENLSEVIKTGKGLIVAWCKQLDVLAHESVGCFVTHCGFNSTLEAISLGVPVVAAPQFSDQTTNAKLLDEILGVGVRVKADENGIVRRGNLASCIKMIMEEERGVIIRKNAVKWKDLAKVAVHEGGSSDNDIVEFVSELIKA

SEQ ID NO: 21 - DNA, 1503 bp, synthetic construct
  source 1..1503: mol_type = other DNA
  misc_feature 1..1503: note = Hydroxymethylglutaryl-CoA reductase from Yarrowia lipolytica, CpO for expression in Yarrowia lipolitica
atgacccagtctgtgaaggtggttgagaagcacgttcctatcgtcattgagaagcccagcgagaaggaggaggacacctcttctgaagactccattgagctgactgtcggaaagcagcccaagcccgtgaccgagacccgttctctggacgacttggaggctatcatgaaggcaggtaagaccaagctcctggaggaccacgaggttgtcaagctctctctcgaaggcaagctccctttgtatgctcttgagaagcagcttggtgacaacacccgagctgttggcatccgacgatctatcatctcccagcagtctaataccaagactcttgagacctcaaagctcccttacctgcactacgactacgaccgtgtttttggagcctgttgcgagaacgttattggttacatgcctctccccgttggtgttgctggccccatgaacattgatggcaagaactaccacattcctatggccaccactgagggttgtcttgttgcctcaaccatgcgaggttgcaaggccatcaacgccggtggcggtgttaccactgtgcttactcaggacggtatgacacgaggtccttgtgtttccttcccctctctcaagcgggctggagccgctaagatctggcttgattccgaggagggtctcaagtccatgcgaaaggccttcaactccacctctcgatttgctcgtctccagtctcttcactctacccttgctggtaacctgctgtttattcgattccgaaccaccactggtgatgccatgggcatgaacatgatctccaagggcgtcgaacactctctggccgtcatggtcaaggagtacggcttccctgatatggacattgtgtctgtctcgggtaactactgcactgacaagaagcccgcagcgatcaactggatcgaaggccgaggcaagagtgttgttgccgaagccaccatccctgctcacattgtcaagtctgttctcaaaagtgaggttgacgctcttgttgagctcaacatcagcaagaatctgatcggtagtgccatggctggctctgtgggaggtttcaatgcacacgccgcaaacctggtgaccgccatctaccttgccactggccaggatcctgctcagaatgtcgagtcttccaactgcatcacgctgatgagcaacgtcgacggtaacctgctcatctccgtttccatgccttctatcgaggtcggtaccattggtggaggtactattttggagccccagggtgctatgctggagatgcttggcgtgcgaggtcctcacatcgagacccccggtgccaacgcccaacagcttgctcgcatcattgcttctggagttcttgcagcggagctttcgctgtgttctgctcttgctgccggccatcttgtgcaaagtcatatgacccacaaccgttcccaggctcctactccggccaagcagtctcaggccgatctgcagcgtctccaaaacggttcgaatatctgcattcggtcatag

SEQ ID NO: 22 - DNA, 984 bp, synthetic construct
  source 1..984: mol_type = other DNA
  misc_feature 1..984: note = Geranylgeranyl diphosphate synthase from Yarrowia lipolytica CpO for expression in Yarrowia lipolytica
atggattataacagcgcggatttcaaggagatctggggcaaggccgccgacaccgcgctgctgggaccgtacaactacctcgccaacaaccggggccacaacatcagagaacacttgatcgcagcgttcggagcggttatcaaggtggacaagagcgatctcgaaaccatttcgcacatcaccaagattttgcataactcgtcgctgcttgttgatgacgtggaagacaactcgatgctccgacgaggcctgccggcagcccattgtctgtttggagtcccccaaaccatcaactccgccaactacatgtactttgtggctctgcaggaggtgctcaagctcaagtcttatgatgccgtctccattttcaccgaggaaatgatcaacttgcatagaggtcagggtatggatctctactggagagaaacactcacttgcccctcggaagacgagtatctggagatggtggtgcacaagaccggaggactgtttcggctggctctgagacttatgctgtcggtggcatcgaaacaggaggaccatgaaaagatcaactttgatctcacacaccttaccgacacactgggagtcatttaccagattctggatgattacctcaacctgcagtccacggaattgaccgagaacaagggattctgcgaagatatcagcgaaggaaagttttcgtttccgctgattcacagcatccggaccaacccggataaccacgagattctcaacattctcaaacagcgaacaagcgacgcttcactcaaaaagtacgccgtggactacatgagaacagaaaccaagagtttcgactactgcctcaagagaatccaggccatgtcactcaaggcaagttcgtacattgatgatctcgcagcagccggccacgatgtctccaagttgcgagccattttgcattattttgtgtccacctctgactgtgaggagagaaagtactttgaggatgcgcagtga

SEQ ID NO: 23 - DNA, 2232 bp, synthetic construct
  source 1..2232: mol_type = other DNA
  misc_feature 1..2232: note = Copalyl pyrophosphate synthase from Stevia rebaudiana CpO for expression in Yarrowia lipolytica
atgtgcaaggctgtttccaaggagtactccgatctgctccagaaggacgaggcctctttcaccaagtgggacgacgacaaggtcaaggaccacctcgacaccaacaagaacctctaccccaacgacgagatcaaggagtttgtcgagtccgtcaaggccatgttcggctccatgaacgacggcgagattaatgtctctgcttacgacaccgcctgggttgctctggtccaggatgtcgacggttccggctctcctcagttcccttcctctctcgagtggatcgccaacaaccagctgtccgacggttcttggggtgaccacctgctcttctctgctcacgaccgaatcatcaacaccctggcctgtgtcattgctctgacctcttggaacgtccacccctccaagtgcgagaagggtctgaacttcctccgagagaacatctgcaagctcgaggacgagaacgccgagcacatgcccattggcttcgaggtcaccttcccctctctgattgacattgccaagaagctcaacattgaggtccccgaggacacccccgctctcaaggagatctacgctcgacgagacatcaagctcaccaagatccccatggaggttctccacaaggtccccaccactctcctccactctctcgagggtatgcccgatctcgagtgggagaagctgctcaagctgcagtgcaaggacggctctttcctcttctccccctcttccactgccttcgccctcatgcagaccaaggacgagaagtgtctccagtacctcaccaacattgtcaccaagttcaacggtggtgtccccaacgtctaccccgttgacctctttgagcacatctgggttgttgaccgactccagcgactcggtatcgcccgatacttcaagtccgagatcaaggactgtgtcgagtacatcaacaagtactggaccaagaacggtatctgctgggcccgaaacacccacgtccaggacattgacgacaccgccatgggcttccgagttctgcgagcccacggctacgatgtcacccccgatgtctttcgacagtttgagaaggacggcaagtttgtctgtttcgccggtcagtccacccaggccgtcaccggtatgttcaacgtctaccgagcttctcagatgctcttccccggtgagcgaatcctcgaggacgccaagaagttctcctacaactacctcaaggagaagcagtccaccaacgagctgctcgacaagtggatcattgccaaggatctgcccggtgaggttggctacgccctcgacatcccctggtacgcctctctgccccgactggagactcgatactacctcgagcagtacggtggtgaggacgatgtctggatcggtaagaccctgtaccgaatgggctacgtttccaacaacacctacctcgagatggccaagctcgactacaacaactacgttgccgtcctccagctcgagtggtacaccatccagcagtggtacgtcgacattggtatcgagaagttcgagtccgacaacatcaagtccgtccttgtctcctactacctcgctgctgcctccatcttcgagcccgagcgatccaaggagcgaattgcctgggccaagaccaccatcctcgtcgacaagatcacctccatcttcgactcctcccagtcctccaaggaagatatcaccgccttcattgacaagttccgaaacaagtcctcctccaagaagcactccatcaacggcgagccctggcacgaggtcatggttgctctcaagaaaactctccacggctttgccctcgacgctctgatgacccactctcaggacatccacccccagctccaccaggcctgggagatgtggctcaccaagctccaggacggtgttgatgtcactgctgagctcatggtccagatgatcaacatgaccgccggccgatgggtttccaaggagctcctcacccacccccagtaccagcgactctccactgtcaccaactctgtctgccacgacatcaccaagctccacaacttcaaggagaactccaccaccgtcgactccaaggtccaggagctggtccagctcgttttctccgacacccccgatgatctcgaccaggacatgaagcagaccttcctgactgtcatgaaaactttctactacaaggcctggtgcgaccccaacaccatcaacgaccacatctccaaggtctttgagattgtgatttaa

SEQ ID NO: 24 - DNA, 2274 bp, synthetic construct
  source 1..2274: mol_type = other DNA
  misc_feature 1..2274: note = Kaurene synthase from Stevia rebaudiana CpO for expression in Yarrowia lipolytica
atgacctcccacggcggccagaccaaccccaccaacctcatcattgacaccaccaaggagcgaatccagaagcagttcaagaacgtcgagatctccgtttcctcctacgacaccgcctgggtcgccatggtcccctctcccaactcccccaagtctccctgcttccccgagtgtctcaactggctcatcaacaaccagctcaacgacggctcttggggtctggtcaaccacacccacaaccacaaccaccccctcctcaaggactctctctcttccactctcgcctgcattgttgctctcaagcgatggaacgttggcgaggaccagatcaacaagggtctgtctttcattgagtccaacctcgcctccgccaccgagaagtcccagccctcccccattggctttgatatcatcttccccggtctgctcgagtacgccaagaacctcgatatcaacctgctctccaagcagaccgacttctctctcatgctgcacaagcgagagctcgagcagaagcgatgccactccaacgagatggacggctacctggcctacatttccgagggtctgggtaacctctacgactggaacatggtcaagaagtaccagatgaagaacggttccgttttcaactccccctctgccaccgctgctgccttcatcaaccaccagaaccccggctgtctcaactacctcaactctctgctcgacaagtttggtaacgccgtccccactgtctacccccacgatctcttcatccgactctccatggtcgacaccattgagcgactcggtatttcccaccacttccgagtcgagatcaagaacgttctcgatgagacttaccgatgctgggttgagcgagatgagcagatcttcatggacgttgtcacctgtgctctggccttccgactcctccgaatcaacggttacgaggtttcccccgaccccctcgccgagatcaccaacgagctggctctcaaggacgagtacgccgccctcgagacttaccacgcttctcacattctgtaccaagaggatctgtcctccggcaagcagattctcaagtccgccgacttcctcaaggagatcatctccactgactccaaccgactctccaagctcatccacaaggaagtcgagaacgctctcaagttccccatcaacaccggtctggagcgaatcaacacccgacgaaacatccagctctacaacgtcgacaacacccgaattctcaagaccacctaccactcttccaacatctccaacaccgactacctgcgactcgccgtcgaggacttctacacctgccagtccatctaccgagaggagctcaagggtctggagcgatgggttgtcgagaacaagctcgaccagctcaagtttgcccgacaaaagactgcctactgctacttctccgttgctgccaccctctcttctcccgagctctccgacgcccgaatctcttgggccaagaacggtatcctgaccactgttgtcgacgacttctttgacattggtggcaccattgacgagctgaccaacctcatccagtgcgtcgagaagtggaacgtcgacgttgacaaggactgttgttccgagcacgtccgaatcctcttcctggctctcaaggacgccatctgctggatcggtgacgaggccttcaagtggcaggctcgagatgtcacttcccacgtcatccagacctggctcgagctcatgaactccatgctgcgagaggccatctggacccgagatgcctacgtccccaccctcaacgagtacatggagaacgcctacgtcagctttgctctcggtcccattgtcaagcccgccatctactttgtcggtcccaagctgtccgaggagattgtcgagtcctccgagtaccacaacctcttcaagctcatgtccacccagggccgactcctcaacgatatccactccttcaagcgagagttcaaggaaggtaagctcaacgccgttgctctgcacctgtccaacggtgagtccggcaaggtcgaggaagaggtcgtcgaggagatgatgatgatgatcaagaacaagcgaaaggagctcatgaagctcatcttcgaggagaacggctccattgtcccccgagcctgcaaggacgccttctggaacatgtgccacgtcctcaacttcttctacgccaacgacgacggtttcaccggcaacaccattctcgacaccgtcaaggacatcatctacaaccctctggttctggtcaacgagaacgaggagcagaggtaa

SEQ ID NO: 25 - DNA, 1578 bp, synthetic construct
  source 1..1578: mol_type = other DNA
  misc_feature 1..1578: note = Kaurene oxidase from Giberella fujikuroi CpO for expression in Yarrowia lipolytica
atgtccaagtccaactccatgaactccacctcccacgagactctcttccagcagctcgttctcggcctcgaccgaatgcccctcatggacgtccactggctcatctacgttgcctttggtgcctggctctgctcctacgtcatccacgttctgtcctcttcctccactgtcaaggtccccgtcgtcggttaccgatccgttttcgagcccacctggctcctccgactgcgattcgtctgggagggtggttccatcattggccagggctacaacaagttcaaggactccatcttccaggtccgaaagctcggtaccgacattgtcatcatccctcccaactacattgacgaggtccgaaagctctcccaggacaagacccgatccgtcgagcccttcatcaacgactttgccggccagtacacccgaggtatggtctttctgcagtccgatctccagaaccgagtcatccagcagcgactcacccccaagcttgtctctctcaccaaggtcatgaaggaagagctcgactacgctctgaccaaggagatgcccgacatgaagaacgacgagtgggttgaggtcgacatctcttccatcatggtccgactcatctctcgaatctccgcccgagttttcctcggccccgagcactgccgaaaccaggagtggctcaccaccaccgccgagtactccgagtctctcttcatcaccggcttcatcctccgagttgtcccccacattctccgacccttcattgctcctctgctgccctcttaccgaaccctgctgcgaaacgtttcttccggccgacgagtcattggtgatatcatccgatcccagcagggtgacggtaacgaggacatcctctcttggatgcgagatgctgccactggtgaggagaagcagatcgacaacattgcccagcgaatgctcattctgtctctcgcctccatccacaccaccgccatgaccatgacccacgccatgtacgatctgtgtgcctgccccgagtacattgagcccctccgagatgaggtcaagtccgtcgttggtgcttctggctgggacaagaccgctctcaaccgattccacaagctcgactctttcctcaaggagtcccagcgattcaaccccgttttcctgctcaccttcaaccgaatctaccaccagtccatgaccctctccgatggtaccaacatcccctccggtacccgaattgctgtcccctctcacgccatgctccaggactccgcccacgtccccggtcccactcctcccactgagttcgacggtttccgatactccaagatccgatccgactccaactacgcccagaagtacctcttctccatgaccgactcttccaacatggcctttggctacggtaagtacgcctgccccggccgattctacgcctccaacgagatgaagctgactctggccattctgctcctccagtttgagttcaagctccccgacggtaagggccgaccccgaaacatcaccatcgactccgacatgatccccgacccccgagctcgactctgtgtccgaaagcgatctctgcgtgacgagtaa

SEQ ID NO: 26 - DNA, 1578 bp, synthetic construct
  source 1..1578: mol_type = other DNA
  misc_feature 1..1578: note = Kaurenoic acid 13-hydroxylase from Arabidopsis thaliana, codon-pair optimized for expression in Yarrowia lipolytica
atggagtctctggttgtccacaccgtcaacgccatctggtgcattgtcattgtcggtatcttctccgtcggctaccacgtctacggccgagctgttgtcgagcagtggcgaatgcgacgatctctcaagctccagggtgtcaagggtcctcctccctccatcttcaacggtaacgtttccgagatgcagcgaatccagtccgaggccaagcactgctccggtgacaacatcatctcccacgactactcttcttctctgttcccccactttgaccactggcgaaagcagtacggccgaatctacacctactccactggcctcaagcagcacctctacatcaaccaccccgagatggtcaaggagctctcccagaccaacaccctcaacctcggccgaatcacccacatcaccaagcgactcaaccccattctcggtaacggtatcatcacctccaacggcccccactgggcccaccagcgacgaatcattgcctacgagttcacccacgacaagatcaagggtatggtcggtctgatggtcgagtccgccatgcccatgctcaacaagtgggaggagatggtcaagcgaggtggtgagatgggctgtgacatccgagtcgacgaggacctcaaggatgtctccgctgacgtcattgccaaggcctgtttcggctcttccttctccaagggcaaggccatcttctccatgatccgagatctgctcaccgccatcaccaagcgatccgtcctcttccgattcaacggtttcaccgacatggttttcggctccaagaagcacggtgacgttgacattgacgctctcgagatggagctcgagtcctccatctgggagactgtcaaggagcgagagattgagtgcaaggacacccacaagaaggacctcatgcagctcattctcgagggtgccatgcgatcttgtgacggtaacctgtgggacaagtctgcttaccgacgattcgttgtcgacaactgcaagtccatctactttgccggccacgactccaccgccgtttccgtttcttggtgcctcatgctgctcgctctcaacccctcttggcaggtcaagatccgagatgagattctgtcctcctgcaagaacggtatccccgacgccgagtccatccccaacctcaagaccgtcaccatggtcatccaggagactatgcgactctaccctcccgctcccattgtcggccgagaggcctccaaggacattcgactcggtgatctggttgtccccaagggtgtctgtatctggaccctcatccccgctctgcaccgagatcccgagatctggggtcccgacgccaacgacttcaagcccgagcgattctccgagggtatctccaaggcctgcaagtacccccagtcctacatcccctttggcctcggcccccgaacctgtgtcggcaagaactttggtatgatggaggtcaaggtcctcgtttctctgattgtctccaagttctccttcactctgtctcccacctaccagcactctccctcccacaagctgctcgtcgagccccagcacggtgttgtcatccgagttgtataa

SEQ ID NO: 27 - DNA, 2136 bp, synthetic construct
  source 1..2136: mol_type = other DNA
  misc_feature 1..2136: note = Cytochrome P450 reductase from Arabidopsis thaliana CpO for expression in Yarrowia lipolytica
atgtcctcctcttcttcttcttccacctccatgattgatctcatggctgccatcatcaagggtgagcccgtcattgtctccgaccccgccaacgcctccgcctacgagtccgttgctgccgagctgtcctccatgctcatcgagaaccgacagtttgccatgatcgtcaccacctccattgctgttctcattggctgcattgtcatgctcgtctggcgacgatctggctccggtaactccaagcgagtcgagcccctcaagcccctggtcatcaagccccgagaagaggagatcgacgacggccgaaagaaggtcaccatcttctttggcacccagaccggtactgctgagggcttcgccaaggctctcggtgaggaagccaaggctcgatacgaaaagacccgattcaagattgtcgacctcgatgattacgctgccgatgacgacgagtacgaggagaagctcaagaaagaggacgttgccttcttcttcctcgccacctacggtgacggtgagcccaccgacaacgctgcccgattctacaagtggttcaccgagggtaacgaccgaggcgagtggctcaagaacctcaagtacggtgttttcggtctgggcaaccgacagtacgagcacttcaacaaggttgccaaggttgtcgacgacatcctcgtcgagcagggtgcccagcgactcgtccaggtcggcctcggtgatgatgaccagtgcatcgaggacgacttcactgcctggcgagaggctctgtggcccgagctcgacaccattctgcgagaggaaggtgacaccgccgttgccaccccctacaccgccgccgtcctcgagtaccgagtctccatccacgactccgaggatgccaagttcaacgacatcaacatggccaacggtaacggctacaccgtctttgacgcccagcacccctacaaggccaacgtcgccgtcaagcgagagctccacacccccgagtccgaccgatcttgtatccacctcgagtttgacattgctggttccggtctgacctacgagactggtgaccacgttggtgtcctctgtgacaacctgtccgagactgtcgacgaggctctgcgactcctcgacatgtcccccgacacttacttctctctgcacgccgagaaagaggacggtactcccatctcttcttctctgccccctcccttccctccctgcaacctgcgaaccgctctgacccgatacgcctgcctcctctcttctcccaagaagtctgctctcgttgctctggccgcccacgcctccgaccccaccgaggctgagcgactcaagcacctcgcctctcccgctggcaaggacgagtactccaagtgggttgtcgagtcccagcgatctctgctcgaggtcatggccgagttcccctccgccaagccccctctcggtgttttcttcgccggtgttgctccccgactccagccccgattctactccatctcctcttcccccaagatcgccgagactcgaatccacgttacctgtgctctggtctacgagaagatgcccaccggccgaatccacaagggtgtctgctccacctggatgaagaacgccgttccctacgagaagtccgagaactgttcctctgctcccatctttgtccgacagtccaacttcaagctcccctccgactccaaggtccccatcatcatgattggccccggtaccggcctcgcccccttccgaggcttcctgcaggagcgactcgccctcgtcgagtccggtgtcgagctcggcccctccgtcctcttctttggctgccgaaaccgacgaatggacttcatctacgaagaggagctccagcgattcgtcgagtccggtgctctcgccgagctctccgttgccttctcccgagagggtcccaccaaggagtacgtccagcacaagatgatggacaaggcctccgacatctggaacatgatctcccagggcgcctacctctacgtctgcggtgacgccaagggtatggcccgagatgtccaccgatctctgcacaccattgcccaggagcagggctccatggactccaccaaggccgagggtttcgtcaagaacctccagacctccggccgatacctccgagatgtctggtaa

SEQ ID NO: 28 - DNA, 1446 bp, synthetic construct
  source 1..1446: mol_type = other DNA
  misc_feature 1..1446: note = UDP-glycosyltransferase from Stevia rebaudiana Cpo for expression in Yarrowia lipolytica
atggacgccatggccaccaccgagaagaagccccacgtcatcttcatccccttccccgcccagtcccacatcaaggccatgctcaagctcgcccagctcctccaccacaagggcctccagatcacctttgtcaacaccgacttcatccacaaccagttcctcgagtcctccggcccccactgtctggacggtgctcccggtttccgatttgagactatccccgatggtgtctcccactcccccgaggcctccatccccatccgagagtctctgctccgatccattgagactaacttcctcgaccgattcattgatctcgtcaccaagctccccgatcctcccacctgtatcatctccgacggtttcctgtccgttttcaccattgatgctgccaagaagctcggtatccccgtcatgatgtactggactctggctgcctgtggtttcatgggtttctaccacatccactctctgatcgagaagggctttgctcctctcaaggacgcctcctacctcaccaacggttacctcgacaccgtcattgactgggtccccggtatggagggtatccgactcaaggacttccccctcgactggtccaccgacctcaacgacaaggttctcatgttcaccaccgaggctccccagcgatcccacaaggtttcccaccacatcttccacaccttcgacgagctcgagccctccatcatcaagactctgtctctgcgatacaaccacatctacaccattggccccctccagctcctcctcgaccagatccccgaggagaagaagcagaccggtatcacctctctgcacggctactctctcgtcaaggaagagcccgagtgcttccagtggctccagtccaaggagcccaactccgttgtctacgtcaactttggctccaccaccgtcatgtctctcgaggacatgaccgagtttggctggggtctggccaactccaaccactacttcctgtggatcatccgatccaacctcgtcattggcgagaacgccgttctgcctcccgagctcgaggagcacatcaagaagcgaggcttcattgcctcttggtgctcccaggagaaggttctcaagcacccctccgtcggtggtttcctgacccactgcggctggggctccaccattgagtctctgtccgctggtgtccccatgatctgctggccctactcctgggaccagctcaccaactgccgatacatctgcaaggagtgggaggttggtctggagatgggtaccaaggtcaagcgagatgaggtcaagcgactcgtccaggagctcatgggcgagggtggtcacaagatgcgaaacaaggccaaggactggaaggagaaggcccgaattgccattgcccccaacggctcttcttctctcaacattgacaagatggtcaaggagatcactgttctcgctcgaaactaa

SEQ ID NO: 29 - DNA, 1422 bp, synthetic construct
  source 1..1422: mol_type = other DNA
  misc_feature 1..1422: note = Variant of UDP-glycosyltransferase from Stevia rebaudiana Cpo for expression in Yarrowia lipolytica
atggccacctccgactccattgttgacgaccgaaagaagctccacattgtcatgttcccctggctcgcctttggccacatcatcccctatctcgagctttccaagctcattgcccagaagggccacaaggtttccttcctctccaccaccaagaacattgaccgactctcctcccacatctctcccctcatcaactttgtcaagctcaccctcccccgagtccaggagctgcccgaggacgccgaggccaccactgatgtccaccccgaggatatcccctacctcaagaaggcctccgacggcctccagcccgaggtcactgagttcctcgagcagcactctcccgactggatcatctacgactacacccactactggctccccgagattgccaagtctctcggtgtctctcgagcccacttctccgtcaccaccccctgggccattgcttacatgggtcccactgccgatgccatgatcaacggttccgactaccgaaccgagcttgaggacttcaccgtccctcccaagtggttccccttccccaccaccgtctgctggcgaaagcacgatctggcccgactcgtcccctacaaggctcccggtatctccgacggttaccgaatgggcctcgtcatcaagggctgcgactgtctgctctccaagacctaccacgagttcggtactcagtggctccgacttctcgaggagctgcaccgagtccccgtcatccccgttggtctgctccctccctccatccccggctctgacaaggacgactcttgggtttccatcaaggagtggctcgacggccaggagaagggctccgttgtctacgttgctctcggttccgaggttctcgtcacccaggaagaggttgtcgagcttgctcacggtctggagctgtccggtctgcccttcttctgggcctaccgaaagcccaagggtcccgccaagtccgactccgtcgagcttcccgatggtttcgtcgagcgagtccgagatcgaggtctggtctggacctcttgggctccccagctccgaatcctctcccacgagtccgttgctggtttcctcacccactgcggttccggctccattgtcgagggcctcatgttcggccaccctctcatcatgctccccatcttcggtgaccagcccctcaacgcccgactccttgaggacaagcaggtcggtatcgagatcccccgaaacgaggaagatggttctttcacccgagactctgttgccgagtctctgcgactcgtcatggtcgaggaagagggtaagatctaccgagagaaggccaaggagatgtccaagctctttggcgacaaggacctccaggaccagtacgtcgacgactttgtcgagtacctccagaagcaccgacgagctgttgccattgaccacgaaagctaa

SEQ ID NO: 30 - DNA, 1377 bp, synthetic construct
  source 1..1377: mol_type = other DNA
  misc_feature 1..1377: note = UDP-glycosyltransferase from Stevia rebaudiana Cpo for expression in Yarrowia lipolytica
atggagaacaagaccgagactaccgtccgacgacgacgacgaatcattctcttccccgtccccttccagggccacatcaaccccattctgcagctcgccaacgttctgtactccaagggcttctccatcaccatcttccacaccaacttcaacaagcccaagacctccaactacccccacttcactttccgattcatcctcgacaacgacccccaggacgagcgaatctccaacctgcccacccacggtcctctggctggtatgcgaatccccatcatcaacgagcacggtgctgacgagctccgacgagagctcgagctgctcatgctcgcctccgaagaggacgaggaagtctcctgtctgatcaccgatgctctgtggtactttgcccagtccgtcgccgactctctcaacctgcgacgactcgttctcatgacctcctctctgttcaacttccacgcccacgtttctctgccccagtttgacgagctcggttacctcgaccccgatgacaagacccgactcgaggagcaggcttccggtttccccatgctcaaggtcaaggacatcaagtccgcctactccaactggcagattctcaaggagattctcggcaagatgatcaagcagaccaaggcctcctccggtgtcatctggaactccttcaaggagctcgaggagtccgagctcgagactgtcatccgagagatccccgctccctctttcctcatccccctgcccaagcacctcaccgcttcctcctcttctctgctcgaccacgaccgaaccgtctttcagtggctcgaccagcagcccccttcctccgtcctctacgtttccttcggctccacctccgaggtcgacgagaaggacttcctcgagattgctcgaggcctcgttgactccaagcagtccttcctgtgggttgtccgacccggctttgtcaagggctccacctgggttgagcccctgcccgatggtttcctcggtgagcgaggccgaattgtcaagtgggtcccccagcaggaagttctggcccacggtgccattggtgccttctggacccactccggctggaactccactctcgagtccgtctgcgagggtgtccccatgatcttctccgactttggcctcgaccagcccctcaacgcccgatacatgtccgatgttctcaaggtcggtgtctacctcgagaacggctgggagcgaggtgagattgccaacgccatccgacgagtcatggtcgacgaggaaggtgagtacatccgacagaacgcccgagtcctcaagcagaaggccgatgtctctctcatgaagggtggttcttcttacgagtctctcgagtctctcgtttcctacatctcttctttgtaa

SEQ ID NO: 31 - DNA, 999 bp, synthetic construct
  source 1..999: mol_type = other DNA
  misc_feature 1..999: note = HSP promoter
gtgcaatcacatgttgctactgtacctgctgtggaccacgcacggcggaacgtaccgtacaaatattttcttgctcacatgactctctctcggccgcgcacgccggtggcaaattgctcttgcattggctctgtctctagacgtccaaaccgtccaaagtggcagggtgacgtgatgcgacgcacgaaggagatggcccggtggcgaggaaccggacacggcgagccggcgggaaaaaaggcggaaaacgaaaagcgaagggcacaatctgacggtgcggctgccaccaacccaaggaggctattttgggtcgctttccatttcacattcgccctcaatggccactttgcggtggtgaacatggtttctgaaacaaccccccagaattagagtatattgatgtgtttaagattgggttgctatttggccattgtgggggagggtagcgacgtggaggacattccagggcgaattgagcctagaaagtggtagcattccaaccgtctaagtcgtccgaattgatcgctataactatcacctctctcacatgtctacttccccaaccaacatccccaacctcccccacactaaagttcacgccaataatgtaggcactctttctgggtgtgggacagcagagcaatacggaggggagattacacaacgagccacaattggggagatggtagccatctcactcgacccgtcgacttttggcaacgctcaattacccaccaaatttgggctggagttgaggggaccgtgttccagcgctgtaggaccagcaacacacacggtatcaacagcaaccaacgcccccgctaatgcacccagtactgcgcaggtgtgggccaggtgcgttccagatgcgagttggcgaaccctaagccgacagtgtactttttgggacgggcagtagcaatcgtgggcggaaaccccggtgtatataaaggggtggagaggacggattattagcaccaacacacacacttatactac

SEQ ID NO: 32 - DNA, 300 bp, synthetic construct
  source 1..300: mol_type = other DNA
  misc_feature 1..300: note = Pgm terminator
acttcgagctaatccagtagcttacgttacccaggggcaggtcaactggctagccacgagtctgtcccaggtcgcaatttagtgtaataaacaatatatatattgagtctaaagggaattgtagctattgtgattgtgtgattttcgtcttgctggttcttattgtgtcccattcgtttcatcctgatgaggacccctggaaccggtgttttcttagtctctgcaatcgctagtcttgttgctatgacagttgcgtcgacactattcaggtcatctatcggttattctgatattataata

SEQ ID NO: 33 - DNA, 403 bp, synthetic construct
  source 1..403: mol_type = other DNA
  misc_feature 1..403: note = pAgos_lox TEF1 promoter
taccgttcgtataatgtatgctatacgaagttatgtccccgccgggtcacccggccagcgacatggaggcccagaataccctccttgacagtcttgacgtgcgcagctcaggggcatgatgtgactgtcgcccgtacatttagcccatacatccccatgtataatcatttgcatccatacattttgatggccgcacggcgcgaagcaaaaattacggctcctcgctgcagacctgcgagcagggaaacgctcccctcacagacgcgttgaattgtccccacgccgcgcccctgtagagaaatataaaaggttaggatttgccactgaggttcttctttcatatacttccttttaaaatcttgctaggatacagttctcacatcacatccgaacataaacaaca

SEQ ID NO: 34 - DNA, 285 bp, synthetic construct
  source 1..285: mol_type = other DNA
  misc_feature 1..285: note = Agos tef1Ts_lox terminator
atcagtactgacaataaaaagattcttgttttcaagaacttgtcatttgtatagtttttttatattgtagttgttctattttaatcaaatgttagcgtgatttatattttttttcgcctcgacatcatctgcccagatgcgaagttaagtgcgcagaaagtaatatcatgcgtcaatcgtatgtgaatgctggtcgctatactgctgtcgattcgatactaacgccgccatccagtgtcgaaaacgagctcataacttcgtataatgtatgctatacgaacggta